European Patent Application EP 4 306 539 A1, published January 17, 2024. Title: ANTI-VRICELLA-ZOSTER VIRUS ANTIBODY AND USE THEREOF. Applicant: BEIJING WISDOMAB BIOTECHNOLOGY CO.,LTD GENRIX (SHANGHAI) BIOPHARMACEUTICAL CO., LTD CHONGQING GENRIX BIOPHARMACEUTICAL CO., LTD. Application EP 22766092.5. The sequence listing filed with the application follows.

SEQUENCE LISTING (28 sequences)

SEQ ID NO: 1 - protein, 118 aa, Artificial Sequence
  Synthetic Polypeptide
QVQLKESGPGPVKPSQSLSLTCSVTGYSITSGNYWNWVRQFPGNKLEWMAYISYDGSTYYNPSLKNRISITRDTSKNQFFLKLNSVTTEDTATYYCAEGYYGYWFAYWGQGTLVTVSA

SEQ ID NO: 2 - protein, 106 aa, Artificial Sequence
  Synthetic Polypeptide
ENVLTQSPAILSASPGEKVTMTCRASSSVSYMHWYQQKPGSSPKPWIYATSNLASGVPARFSGSGSGTSYSLTISRVEAEDAATYYCQQWSSNPFTFGSGTKLEIK

SEQ ID NO: 3 - protein, 121 aa, Artificial Sequence
  Synthetic Polypeptide
EVKLVESGPGLVKPSQSLSLTCSVTGYSITSGYYWNWIRQFPGNKLEWMGYISYDGSNNYNTSLKNRISITRDTSKNQFFLKLNSVTTEDTATYYCAREDVNYPPYALDYWGQGTSVTVSS

SEQ ID NO: 4 - protein, 112 aa, Artificial Sequence
  Synthetic Polypeptide
SIVMTQTPLSLPVSLGDQASISCRSSQSLVHSNGNTYLHWYLQKPGQSPKLLIYKVSNRFSGVPDRFSGSGSGTDFTLKISRVEAEDLGVYFCSQSTHVPWTFGGGTKLEMK

SEQ ID NO: 5 - protein, 118 aa, Artificial Sequence
  Synthetic Polypeptide
EVKLVESGGGLVQPGGSLKLSCAASGFTFSSYTMSWVRQTPEKRLEWVAFISNGGDNNYYADTVKGRFIISRDNAKNTLYLQMSSLKSEDTAMYYCARHNGNWGFAYWGQGTLVTVSA

SEQ ID NO: 6 - protein, 108 aa, Artificial Sequence
  Synthetic Polypeptide
QNVLTQSPTTMAASPGEKITITCSASSSISSNYLHWYQQKPGFSPKLLIYRTSNLASGVPARFSGSGSGTSYSLTIGTMEAEDVATYYCQQGSSIPLTFGAGTKLEIK

SEQ ID NO: 7 - protein, 121 aa, Artificial Sequence
  Synthetic Polypeptide
EVQLVESGGGVVQPGRSLRLSCGASGFTFNTYAMHWVRQAPGKGMEWVAVISYGGGNRYYAASVKGRFTISRDNSKNTLFLQLNTLRPEDTAVYYCARARDNHYFFGMDVWGRGTTVTVSS

SEQ ID NO: 8 - protein, 107 aa, Artificial Sequence
  Synthetic Polypeptide
DIQMTQSPSSVSASVGDRVTITCRASQGISSWLAWYQQKPGKAPKLLIYAASSLQSGVPSRFSGSGSGTDFTLTISSLQPEDFATYYCQEGFYFPINFGGGTKVEIK

SEQ ID NO: 9 - protein, 107 aa, Artificial Sequence
  Synthetic Polypeptide
DIQMTQSPSSVSASVGDRVTITCRASQGISSWLAWYQQKPGKAPKLLIYAASSLQSGVPSRFSGSGSGTDFTLTISSLQPEDFATYYCQQATYFPINFGGGTKVEIK

SEQ ID NO: 10 - protein, 107 aa, Artificial Sequence
  Synthetic Polypeptide
DIQMTQSPSSVSASVGDRVTITCRASQGISSWLAWYQQKPGKAPKLLIYAASSLQSGVPSRFSGSGSGTDFTLTISSLQPEDFATYYCQQSSYFPIAFGGGTKVEIK

SEQ ID NO: 11 - protein, 778 aa, Varicella zoster
NKSYVTPTPATRSIGHMSALLREYSDRNMSLKLEAFYPTGFDEELIKSLHWGNDRKHVFLVIVKVNPTTHEGDVGLVIFPKYLLSPYHFKAEHRAPFPAGRFGFLSHPVTPDVSFFDSSFAPYLTTQHLVAFTTFPPNPLVWHLERAETAATAERPFGVSLLPARPTVPKNTILEHKAHFATWDALARHTFFSAEAIITNSTLRIHVPLFGSVWPIRYWATGSVLLTSDSGRVEVNIGVGFMSSLISLSSGLPIELIVVPHTVKLNAVTSDTTWFQLNPPGPDPGPSYRVYLLGRGLDMNFSKHATVDICAYPEESLDYRYHLSMAHTEALRMTTKADQHDINEESYYHIAARIATSIFALSEMGRTTEYFLLDEIVDVQYQLKFLNYILMRIGAGAHPNTISGTSDLIFADPSQLHDELSLLFGQVKPANVDYFISYDEARDQLKTAYALSRGQDHVNALSLARRVIMSIYKGLLVKQNLNATERQALFFASMILLNFREGLENSSRVLDGRTTLLLMTSMCTAAHATQAALNIQEGLAYLNPSKHMFTIPNVYSPCMGSLRTDLTEEIHVMNLLSAIPTRPGLNEVLHTQLDESEIFDAAFKTMMIFTTWTAKDLHILHTHVPEVFTCQDAAARNGEYVLILPAVQGHSYVITRNKPQRGLVYSLADVDVYNPISVVYLSKDTCVSEHGVIETVALPHPDNLKECLYCGSVFLRYLTTGAIMDIIIIDSKDTERQLAAMGNSTIPPFNPDMHGDDSKAVLLFPNGTVVTLLGFERR

SEQ ID NO: 12 - protein, 138 aa, Varicella zoster
LHLQDDTPLFFGAKPLSDVSLIITEPCVSSVYEAWDYAAPPVSNLSEALSGIVVKTKCPVPEVILWFKDKQMAYWTNPYVTLKGLTQSVGEEHKSGDIRDALLDALSGVWVDSTPSSTNIPENGCVWGADRLFQRVCQ

SEQ ID NO: 13 - protein, 6 aa, Artificial Sequence
  Synthetic Polypeptide
HHHHHH

SEQ ID NO: 14 - protein, 330 aa, Homo sapiens
ASTKGPSVFPLAPSSKSTSGGTAALGCLVKDYFPEPVTVSWNSGALTSGVHTFPAVLQSSGLYSLSSVVTVPSSSLGTQTYICNVNHKPSNTKVDKRVEPKSCDKTHTCPPCPAPELLGGPSVFLFPPKPKDTLMISRTPEVTCVVVDVSHEDPEVKFNWYVDGVEVHNAKTKPREEQYNSTYRVVSVLTVLHQDWLNGKEYKCKVSNKALPAPIEKTISKAKGQPREPQVYTLPPSREEMTKNQVSLTCLVKGFYPSDIAVEWESNGQPENNYKTTPPVLDSDGSFFLYSKLTVDKSRWQQGNVFSCSVMHEALHNHYTQKSLSLSPGK

SEQ ID NO: 15 - protein, 326 aa, Homo sapiens
ASTKGPSVFPLAPCSRSTSESTAALGCLVKDYFPEPVTVSWNSGALTSGVHTFPAVLQSSGLYSLSSVVTVPSSNFGTQTYTCNVDHKPSNTKVDKTVERKCCVECPPCPAPPVAGPSVFLFPPKPKDTLMISRTPEVTCVVVDVSHEDPEVQFNWYVDGVEVHNAKTKPREEQFNSTFRVVSVLTVVHQDWLNGKEYKCKVSNKGLPAPIEKTISKTKGQPREPQVYTLPPSREEMTKNQVSLTCLVKGFYPSDIAVEWESNGQPENNYKTTPPMLDSDGSFFLYSKLTVDKSRWQQGNVFSCSVMHEALHNHYTQKSLSLSPGK

SEQ ID NO: 16 - protein, 327 aa, Homo sapiens
ASTKGPSVFPLAPCSRSTSESTAALGCLVKDYFPEPVTVSWNSGALTSGVHTFPAVLQSSGLYSLSSVVTVPSSSLGTKTYTCNVDHKPSNTKVDKRVESKYGPPCPPCPAPEFLGGPSVFLFPPKPKDTLMISRTPEVTCVVVDVSQEDPEVQFNWYVDGVEVHNAKTKPREEQFNSTYRVVSVLTVLHQDWLNGKEYKCKVSNKGLPSSIEKTISKAKGQPREPQVYTLPPSQEEMTKNQVSLTCLVKGFYPSDIAVEWESNGQPENNYKTTPPVLDSDGSFFLYSRLTVDKSRWQEGNVFSCSVMHEALHNHYTQKSLSLSLGK

SEQ ID NO: 17 - protein, 324 aa, Mus musculus
AKTTPPSVYPLAPGSAAQTNSMVTLGCLVKGYFPEPVTVTWNSGSLSSGVHTFPAVLESDLYTLSSSVTVPSSPRPSETVTCNVAHPASSTKVDKKIVPRDCGCKPCICTVPEVSSVFIFPPKPKDVLTITLTPKVTCVVVDISKDDPEVQFSWFVDDVEVHTAQTQPREEQFNSTFRSVSELPIMHQDWLNGKEFKCRVNSAAFPAPIEKTISKTKGRPKAPQVYTIPPPKEQMAKDKVSLTCMITDFFPEDITVEWQWNGQPAENYKNTQPIMNTNGSYFVYSKLNVQKSNWEAGNTFTCSVLHEGLHNHHTEKSLSHSPGK

SEQ ID NO: 18 - protein, 330 aa, Mus musculus
AKTTAPSVYPLAPVCGDTTGSSVTLGCLVKGYFPEPVTLTWNSGSLSSGVHTFPAVLQSDLYTLSSSVTVTSSTWPSQSITCNVAHPASSTKVDKKIEPRGPTIKPCPPCKCPAPNLLGGPSVFIFPPKIKDVLMISLSPIVTCVVVDVSEDDPDVQISWFVNNVEVHTAQTQTHREDYNSTLRVVSALPIQHQDWMSGKEFKCKVNNKDLPAPIERTISKPKGSVRAPQVYVLPPPEEEMTKKQVTLTCMVTDFMPEDIYVEWTNNGKTELNYKNTEPVLDSDGSYFMYSKLRVEKKNWVERNSYSCSVVHEGLHNHHTTKSFSRTPGK

SEQ ID NO: 19 - protein, 107 aa, Homo sapiens [sequence omitted]

SEQ ID NO: 20 - protein, 106 aa, Homo sapiens
GQPKAAPSVTLFPPSSEELQANKATLVCLISDFYPGAVTVAWKADSSPVKAGVETTTPSKQSNNKYAASSYLSLTPEQWKSHRSYSCQVTHEGSTVEKTVAPTECS

SEQ ID NO: 21 - protein, 107 aa, Mus musculus
RADAAPTVSIFPPSSEQLTSGGASVVCFLNNFYPKDINVKWKIDGSERQNGVLNSWTDQDSKDSTYSMSSTLTLTKDEYERHNSYTCEATHKTSTSPIVKSFNRNEC

SEQ ID NO: 22 - protein, 106 aa, Mus musculus
GQPKSSPSVTLFPPSSEELETNKATLVCTITDFYPGVVTVDWKVDGTPVTQGMETTQPSKQSNNKYMASSYLTLTARAWERHSSYSCQVTHEGHTVEKSLSRADCS

SEQ ID NO: 23 - DNA, 19 bp, Artificial Sequence
  Synthetic Polynucleotide
tgcatttgaactccttgcc

SEQ ID NO: 24 - DNA, 20 bp, Artificial Sequence
  Synthetic Polynucleotide
ccatcaatcttccacttgac

SEQ ID NO: 25 - protein, 239 aa, Artificial Sequence
  Synthetic Polypeptide
QVQLKESGPGPVKPSQSLSLTCSVTGYSITSGNYWNWVRQFPGNKLEWMAYISYDGSTYYNPSLKNRISITRDTSKNQFFLKLNSVTTEDTATYYCAEGYYGYWFAYWGQGTLVTVSAGGGGSGGGGSGGGGSENVLTQSPAILSASPGEKVTMTCRASSSVSYMHWYQQKPGSSPKPWIYATSNLASGVPARFSGSGSGTSYSLTISRVEAEDAATYYCQQWSSNPFTFGSGTKLEIK

SEQ ID NO: 26 - protein, 248 aa, Artificial Sequence
  Synthetic Polypeptide
EVKLVESGPGLVKPSQSLSLTCSVTGYSITSGYYWNWIRQFPGNKLEWMGYISYDGSNNYNTSLKNRISITRDTSKNQFFLKLNSVTTEDTATYYCAREDVNYPPYALDYWGQGTSVTVSSGGGGSGGGGSGGGGSSIVMTQTPLSLPVSLGDQASISCRSSQSLVHSNGNTYLHWYLQKPGQSPKLLIYKVSNRFSGVPDRFSGSGSGTDFTLKISRVEAEDLGVYFCSQSTHVPWTFGGGTKLEMK

SEQ ID NO: 27 - protein, 241 aa, Artificial Sequence
  Synthetic Polypeptide
EVKLVESGGGLVQPGGSLKLSCAASGFTFSSYTMSWVRQTPEKRLEWVAFISNGGDNNYYADTVKGRFIISRDNAKNTLYLQMSSLKSEDTAMYYCARHNGNWGFAYWGQGTLVTVSAGGGGSGGGGSGGGGSQNVLTQSPTTMAASPGEKITITCSASSSISSNYLHWYQQKPGFSPKLLIYRTSNLASGVPARFSGSGSGTSYSLTIGTMEAEDVATYYCQQGSSIPLTFGAGTKLEIK

SEQ ID NO: 28 - protein, 107 aa, Artificial Sequence
  Synthetic Polypeptide
DIQMTQSPSSVSASVGDRVTITCRASQGISSWLAWYQQKPGKAPKLLIYAASSLQSGVPSRFSGSGSGTDFTLTISSLQPEDFATYYCQQANSFPLTFGGGTKVEIK